European Patent Application EP 4 530 291 A1, published April 2, 2025. Title: 바이러스 뉴클레오캡시드를 이용한 목적 단백질 발현 플랫폼. Applicant: 주식회사 백스다임. The sequence listing filed with the application follows.

SEQUENCE LISTING (7 sequences)

SEQ ID NO: 1 - protein, 54 aa, Human immunodeficiency virus 1
QRGNFRNQRKTVKCFNCGKEGHIAKNCRAPRKKGCWRCGREGHQMKDCTERQAN

SEQ ID NO: 2 - DNA, 162 bp, Human immunodeficiency virus 1
  source 1..162: mol_type = genomic DNA
cagcggggaaacttcaggaaccagagaaaaactgtgaagtgcttcaattgcggaaaggagggccacatcgctaagaactgccgcgcccccagaaagaaaggctgctggagatgcggcagagagggccaccagatgaaggactgcacagagagacaggcaaac

SEQ ID NO: 3 - DNA, 162 bp, synthetic construct
  source 1..162: mol_type = other DNA
cagcgtggtaacttccgtaaccagcgtaaaaccgttaaatgcttcaactgcggcaaagaaggccacatcgcgaaaaactgccgtgcgccgcgtaaaaaaggctgctggcgttgcggccgtgaaggccaccagatgaaagattgcaccgaacgtcaggcgaac

SEQ ID NO: 4 - DNA, 711 bp, synthetic construct
  source 1..711: mol_type = other DNA
agtaaaggagaagaacttttcactggagttgtcccaattcttgttgaattagatggtgatgttaatgggcacaaattttctgtcagtggagagggtgaaggtgatgcaacatacggaaaacttacccttaaatttatttgcactactggaaaactacctgttccatggccaacacttgtcactactttctcttatggtgttcaatgcttttcaagatacccagatcatatgaaacggcatgactttttcaagagtgccatgcccgaaggttatgtacaggaaagaactatatttttcaaagatgacgggaactacaagacacgtgctgaagtcaagtttgaaggtgatacccttgttaatagaatcgagttaaaaggtattgattttaaagaagatggaaacattcttggacacaaattggaatacaactataactcacacaatgtatacatcatggcagacaaacaaaagaatggaatcaaagttaacttcaaaattagacacaacattgaagatggaagcgttcaactagcagaccattatcaacaaaatactccaattggcgatggccctgtccttttaccagacaaccattacctgtccacacaatctgccctttcgaaagatcccaacgaaaagagagaccacatggtccttcttgagtttgtaacagctgctgggattacacatggcatggatgaactatacaaa

SEQ ID NO: 5 - protein, 237 aa, synthetic construct
SKGEELFTGVVPILVELDGDVNGHKFSVSGEGEGDATYGKLTLKFICTTGKLPVPWPTLVTTFSYGVQCFSRYPDHMKRHDFFKSAMPEGYVQERTIFFKDDGNYKTRAEVKFEGDTLVNRIELKGIDFKEDGNILGHKLEYNYNSHNVYIMADKQKNGIKVNFKIRHNIEDGSVQLADHYQQNTPIGDGPVLLPDNHYLSTQSALSKDPNEKRDHMVLLEFVTAAGITHGMDELYK

SEQ ID NO: 6 - DNA, 498 bp, synthetic construct
  source 1..498: mol_type = other DNA
aaatcttacaacctgctgggcttcctgcagcgttcctccaacttccagtgccagaagctgctgtggcagctgaacggtcgcctggaatactgcctgaaagatcgtatgaacttcgatatcccggaagaaatcaaacagttgcagcagttccagaaagaagatgcggcgttaaccatctacgaaatgctgcaaaacattttcgctatcttccgtcaggattccagctccaccggctggaacgaaaccatcgttgaaaaccttctggcgaacgtttatcaccagatcaatcatctgaaaaccgtgctggaagagaaactggaaaaagaagacttcacccgtggtaaactgatgtcctcgctgcacctgaagcgttactacggtcgtatcctgcattatctgaaagcgaaagagtacagccactgcgcttggaccattgttcgtgttgaaattctgcgcaatttctacttcatcaaccgtctgaccggttacctgcgtaac

SEQ ID NO: 7 - protein, 166 aa, synthetic construct
KSYNLLGFLQRSSNFQCQKLLWQLNGRLEYCLKDRMNFDIPEEIKQLQQFQKEDAALTIYEMLQNIFAIFRQDSSSTGWNETIVENLLANVYHQINHLKTVLEEKLEKEDFTRGKLMSSLHLKRYYGRILHYLKAKEYSHCAWTIVRVEILRNFYFINRLTGYLRN